European Patent Specification EP 4 019 973 B1, published May 29, 2024. Title: DETECTION METHOD OF MULTIPLE ANALYTES. Applicant: Industrial Technology Research Institute. The sequence listing filed with the application follows.

SEQUENCE LISTING (3 sequences)

SEQ ID NO: 1 - DNA, 30 bp, Artificial Sequence
  AIV probe
gtctacgctgcagtcctcgctcactgggca

SEQ ID NO: 2 - DNA, 33 bp, Artificial Sequence
  AB nucleic acid to be analyzed
aaaaaaaaaaaaaatcctggagctaagtccgta

SEQ ID NO: 3 - DNA, 90 bp, Artificial Sequence
  AIV nucleic acid to be analyzed
caagaccaatcctgtcacctctgactaaggggattttagggtttgtgttcacgctcaccgtgcccagtgagcgaggactgcagcgtagac